European Patent Application EP 4 674 867 A2, published January 7, 2026. Title: ANTIBODY OR ANTIGEN-BINDING FRAGMENT THEREOF BINDING TO Beta-CTx AND KIT THEREOF. Applicant: SHENZHEN MINDRAY BIO-MEDICAL ELECTRONICS CO., LTD. The sequence listing filed with the application follows.

SEQUENCE LISTING (120 sequences)

SEQ ID NO: 1 - protein, 6 aa, synthetic construct
SSAAIN

SEQ ID NO: 2 - protein, 17 aa, synthetic construct
YIYAGSGSTYYASWAKG

SEQ ID NO: 3 - protein, 11 aa, synthetic construct
VRSLSGGDRNL

SEQ ID NO: 4 - protein, 13 aa, synthetic construct
QSSESVSKNDYLA

SEQ ID NO: 5 - protein, 10 aa, synthetic construct
LLIYRASTLA

SEQ ID NO: 6 - protein, 11 aa, synthetic construct
QGGYSRNNDMT

SEQ ID NO: 7 - protein, 6 aa, synthetic construct
SSAAIN

SEQ ID NO: 8 - protein, 17 aa, synthetic construct
YIYAGDDSIYYASWAKG

SEQ ID NO: 9 - protein, 11 aa, synthetic construct
ARSLSGGDRNL

SEQ ID NO: 10 - protein, 13 aa, synthetic construct
QSSESVSKNNYLA

SEQ ID NO: 11 - protein, 10 aa, synthetic construct
LLIYEASKLP

SEQ ID NO: 12 - protein, 11 aa, synthetic construct
QGGYSRNNDMT

SEQ ID NO: 13 - protein, 6 aa, synthetic construct
SSAAIN

SEQ ID NO: 14 - protein, 17 aa, synthetic construct
YIYAGSASTYYATWAKG

SEQ ID NO: 15 - protein, 11 aa, synthetic construct
ARSLSGGDRNL

SEQ ID NO: 16 - protein, 13 aa, synthetic construct
QSSESVTKNNYLA

SEQ ID NO: 17 - protein, 10 aa, synthetic construct
LLIYEASKLA

SEQ ID NO: 18 - protein, 11 aa, synthetic construct
QGGYSRNNDMT

SEQ ID NO: 19 - protein, 6 aa, synthetic construct
SSAAIN

SEQ ID NO: 20 - protein, 17 aa, synthetic construct
YIYAGSGSTYYASWAKG

SEQ ID NO: 21 - protein, 11 aa, synthetic construct
ARSLSGGDRNL

SEQ ID NO: 22 - protein, 13 aa, synthetic construct
QSSENVAKNNYLA

SEQ ID NO: 23 - protein, 10 aa, synthetic construct
LLIYEASKLA

SEQ ID NO: 24 - protein, 11 aa, synthetic construct
QGGYNRNNDMT

SEQ ID NO: 25 - protein, 6 aa, synthetic construct
SSAAIN

SEQ ID NO: 26 - protein, 17 aa, synthetic construct
YIYAGSGSTYYASWAKG

SEQ ID NO: 27 - protein, 11 aa, synthetic construct
ARSLSGGDRNL

SEQ ID NO: 28 - protein, 13 aa, synthetic construct
QSSESVSKNNYLA

SEQ ID NO: 29 - protein, 10 aa, synthetic construct
LLIYEASKLA

SEQ ID NO: 30 - protein, 11 aa, synthetic construct
QGGYSRNNDMT

SEQ ID NO: 31 - protein, 6 aa, synthetic construct
SKYGVN

SEQ ID NO: 32 - protein, 16 aa, synthetic construct
WITSDGITFYASWAKG

SEQ ID NO: 33 - protein, 11 aa, synthetic construct
TRSILSAWDNI

SEQ ID NO: 34 - protein, 13 aa, synthetic construct
QSSKSVYNGNWLS

SEQ ID NO: 35 - protein, 10 aa, synthetic construct
RLIYSASTLA

SEQ ID NO: 36 - protein, 10 aa, synthetic construct
AGGYSGEIDD

SEQ ID NO: 37 - protein, 6 aa, synthetic construct
SSYYVS

SEQ ID NO: 38 - protein, 16 aa, synthetic construct
GINTGGVAYYATWAKG

SEQ ID NO: 39 - protein, 12 aa, synthetic construct
ARHPGGDAGTDL

SEQ ID NO: 40 - protein, 11 aa, synthetic construct
QASQSITKYLA

SEQ ID NO: 41 - protein, 10 aa, synthetic construct
RLIYKTSTLA

SEQ ID NO: 42 - protein, 14 aa, synthetic construct
QNNVPGKITDSYGA

SEQ ID NO: 43 - protein, 8 aa, synthetic construct
STFGMGVS

SEQ ID NO: 44 - protein, 16 aa, synthetic construct
HIYWDDVKRYNPSLKS

SEQ ID NO: 45 - protein, 10 aa, synthetic construct
ARTAGAWFAF

SEQ ID NO: 46 - protein, 10 aa, synthetic construct
SARSTVNYMH

SEQ ID NO: 47 - protein, 7 aa, synthetic construct
DTSKLAS

SEQ ID NO: 48 - protein, 9 aa, synthetic construct
QQWTSNLLT

SEQ ID NO: 49 - protein, 8 aa, synthetic construct
STYGMGIG

SEQ ID NO: 50 - protein, 16 aa, synthetic construct
HIWWDDVKRYDPVLKS

SEQ ID NO: 51 - protein, 12 aa, synthetic construct
ARIPGDGSHSDY

SEQ ID NO: 52 - protein, 16 aa, synthetic construct
RSTQSLVHSNGITYLE

SEQ ID NO: 53 - protein, 7 aa, synthetic construct
RISNRFS

SEQ ID NO: 54 - protein, 9 aa, synthetic construct
FQGSHGPYT

SEQ ID NO: 55 - protein, 8 aa, synthetic construct
STSGMGIG

SEQ ID NO: 56 - protein, 16 aa, synthetic construct
HIWWDDVKRYDPALKS

SEQ ID NO: 57 - protein, 12 aa, synthetic construct
ARIPGDGSHFDY

SEQ ID NO: 58 - protein, 16 aa, synthetic construct
RSSQSLVHSNGITYLE

SEQ ID NO: 59 - protein, 7 aa, synthetic construct
RVSNRFS

SEQ ID NO: 60 - protein, 9 aa, synthetic construct
FQGSHGPYT

SEQ ID NO: 61 - DNA, 18 bp, synthetic construct
  source 1..18: mol_type = other DNA
agtagcgctgcaataaac

SEQ ID NO: 62 - DNA, 51 bp, synthetic construct
  source 1..51: mol_type = other DNA
tacatttatgctggtagtggtagcacatactacgcgagctgggcgaaaggc

SEQ ID NO: 63 - DNA, 33 bp, synthetic construct
  source 1..33: mol_type = other DNA
gtcagaagtttaagtggtggtgatcggaacttg

SEQ ID NO: 64 - DNA, 39 bp, synthetic construct
  source 1..39: mol_type = other DNA
cagtccagtgagagtgtttctaagaatgattacttagcc

SEQ ID NO: 65 - DNA, 30 bp, synthetic construct
  source 1..30: mol_type = other DNA
ctcctgatctacagggcttccactctggca

SEQ ID NO: 66 - DNA, 33 bp, synthetic construct
  source 1..33: mol_type = other DNA
caaggcggttatagtaggaataatgatatgact

SEQ ID NO: 67 - DNA, 18 bp, synthetic construct
  source 1..18: mol_type = other DNA
agtagcgctgcaataaac

SEQ ID NO: 68 - DNA, 51 bp, synthetic construct
  source 1..51: mol_type = other DNA
tacatttatgctggtgatgatagtatatactacgcgagctgggcgaaaggc

SEQ ID NO: 69 - DNA, 33 bp, synthetic construct
  source 1..33: mol_type = other DNA
gccagaagtttgagtggtggtgatcggaacttg

SEQ ID NO: 70 - DNA, 39 bp, synthetic construct
  source 1..39: mol_type = other DNA
cagtccagtgagagtgtttctaagaacaactacttagcc

SEQ ID NO: 71 - DNA, 30 bp, synthetic construct
  source 1..30: mol_type = other DNA
ctcctgatctacgaagcatccaaactgcca

SEQ ID NO: 72 - DNA, 33 bp, synthetic construct; identical to SEQ ID NO: 66
  source 1..33: mol_type = other DNA

SEQ ID NO: 73 - DNA, 18 bp, synthetic construct
  source 1..18: mol_type = other DNA
agtagcgctgcaataaac

SEQ ID NO: 74 - DNA, 51 bp, synthetic construct
  source 1..51: mol_type = other DNA
tacatttatgctggtagtgctagcacatactacgcgacctgggcgaaaggc

SEQ ID NO: 75 - DNA, 33 bp, synthetic construct; identical to SEQ ID NO: 69
  source 1..33: mol_type = other DNA

SEQ ID NO: 76 - DNA, 39 bp, synthetic construct
  source 1..39: mol_type = other DNA
cagtccagtgagagtgttactaagaacaactacttagcc

SEQ ID NO: 77 - DNA, 30 bp, synthetic construct
  source 1..30: mol_type = other DNA
ctcctgatctacgaagcatccaaactggca

SEQ ID NO: 78 - DNA, 33 bp, synthetic construct; identical to SEQ ID NO: 66
  source 1..33: mol_type = other DNA

SEQ ID NO: 79 - DNA, 18 bp, synthetic construct
  source 1..18: mol_type = other DNA
agtagcgctgcaataaat

SEQ ID NO: 80 - DNA, 51 bp, synthetic construct; identical to SEQ ID NO: 62
  source 1..51: mol_type = other DNA

SEQ ID NO: 81 - DNA, 33 bp, synthetic construct
  source 1..33: mol_type = other DNA
gccagaagtttgagtggcggtgatcggaacttg

SEQ ID NO: 82 - DNA, 39 bp, synthetic construct
  source 1..39: mol_type = other DNA
cagtccagtgagaatgttgctaagaacaactacttagcc

SEQ ID NO: 83 - DNA, 30 bp, synthetic construct; identical to SEQ ID NO: 77
  source 1..30: mol_type = other DNA

SEQ ID NO: 84 - DNA, 33 bp, synthetic construct
  source 1..33: mol_type = other DNA
caaggcggttataataggaataatgatatgact

SEQ ID NO: 85 - DNA, 18 bp, synthetic construct
  source 1..18: mol_type = other DNA
agtagcgctgcaataaat

SEQ ID NO: 86 - DNA, 51 bp, synthetic construct; identical to SEQ ID NO: 62
  source 1..51: mol_type = other DNA

SEQ ID NO: 87 - DNA, 33 bp, synthetic construct; identical to SEQ ID NO: 81
  source 1..33: mol_type = other DNA

SEQ ID NO: 88 - DNA, 39 bp, synthetic construct; identical to SEQ ID NO: 70
  source 1..39: mol_type = other DNA

SEQ ID NO: 89 - DNA, 30 bp, synthetic construct; identical to SEQ ID NO: 77
  source 1..30: mol_type = other DNA

SEQ ID NO: 90 - DNA, 33 bp, synthetic construct; identical to SEQ ID NO: 66
  source 1..33: mol_type = other DNA

SEQ ID NO: 91 - DNA, 18 bp, synthetic construct
  source 1..18: mol_type = other DNA
agtaaatatggagtgaac

SEQ ID NO: 92 - DNA, 48 bp, synthetic construct
  source 1..48: mol_type = other DNA
tggattactagtgatggtatcacattctacgcgagctgggcgaaaggc

SEQ ID NO: 93 - DNA, 33 bp, synthetic construct
  source 1..33: mol_type = other DNA
accagaagtatacttagtgcttgggataacatc

SEQ ID NO: 94 - DNA, 39 bp, synthetic construct
  source 1..39: mol_type = other DNA
cagtccagtaagagtgtttataatgggaactggttatcc

SEQ ID NO: 95 - DNA, 30 bp, synthetic construct
  source 1..30: mol_type = other DNA
cgcctgatctattctgcatccactctggca

SEQ ID NO: 96 - DNA, 30 bp, synthetic construct
  source 1..30: mol_type = other DNA
gcaggcggttatagtggtgagattgatgat

SEQ ID NO: 97 - DNA, 18 bp, synthetic construct
  source 1..18: mol_type = other DNA
agtagctactacgtgagc

SEQ ID NO: 98 - DNA, 48 bp, synthetic construct
  source 1..48: mol_type = other DNA
ggcattaatactggtggtgtcgcatactacgcgacctgggcaaaaggc

SEQ ID NO: 99 - DNA, 36 bp, synthetic construct
  source 1..36: mol_type = other DNA
gccagacatcctggtggtgatgctggtaccgacttg

SEQ ID NO: 100 - DNA, 33 bp, synthetic construct
  source 1..33: mol_type = other DNA
caggccagtcagagcattactaaatacttagcc

SEQ ID NO: 101 - DNA, 30 bp, synthetic construct
  source 1..30: mol_type = other DNA
cgcctgatctacaagacatccactctggca

SEQ ID NO: 102 - DNA, 42 bp, synthetic construct
  source 1..42: mol_type = other DNA
caaaacaatgttcctggtaaaattactgacagttatggggct

SEQ ID NO: 103 - DNA, 24 bp, synthetic construct
  source 1..24: mol_type = other DNA
agcacttttggtatgggtgtgagc

SEQ ID NO: 104 - DNA, 48 bp, synthetic construct
  source 1..48: mol_type = other DNA
cacatttactgggatgatgtcaagcgctataatccatccctgaagagc

SEQ ID NO: 105 - DNA, 30 bp, synthetic construct
  source 1..30: mol_type = other DNA
gctcgaaccgctggggcctggtttgctttc

SEQ ID NO: 106 - DNA, 30 bp, synthetic construct
  source 1..30: mol_type = other DNA
agtgccaggtcaactgtaaattacatgcac

SEQ ID NO: 107 - DNA, 21 bp, synthetic construct
  source 1..21: mol_type = other DNA
gacacatccaaactggcttct

SEQ ID NO: 108 - DNA, 27 bp, synthetic construct
  source 1..27: mol_type = other DNA
cagcagtggactagtaatttgctcacg

SEQ ID NO: 109 - DNA, 24 bp, synthetic construct
  source 1..24: mol_type = other DNA
agcacttatggtatgggtataggc

SEQ ID NO: 110 - DNA, 48 bp, synthetic construct
  source 1..48: mol_type = other DNA
cacatttggtgggatgatgtcaagcgctatgatccagtcctgaagagc

SEQ ID NO: 111 - DNA, 36 bp, synthetic construct
  source 1..36: mol_type = other DNA
gctcgcatacctggggatggttcccacagtgactac

SEQ ID NO: 112 - DNA, 48 bp, synthetic construct
  source 1..48: mol_type = other DNA
agatctactcagagccttgtacatagtaatggaatcacctatttagag

SEQ ID NO: 113 - DNA, 21 bp, synthetic construct
  source 1..21: mol_type = other DNA
agaatttccaaccgattttct

SEQ ID NO: 114 - DNA, 27 bp, synthetic construct
  source 1..27: mol_type = other DNA
tttcaaggttcacatggtccgtacacg

SEQ ID NO: 115 - DNA, 24 bp, synthetic construct
  source 1..24: mol_type = other DNA
agcacttctggtatgggtataggc

SEQ ID NO: 116 - DNA, 48 bp, synthetic construct
  source 1..48: mol_type = other DNA
cacatttggtgggatgatgtcaagcgctatgatccagccctgaagagc

SEQ ID NO: 117 - DNA, 36 bp, synthetic construct
  source 1..36: mol_type = other DNA
gctcgaatacctggggatggttcccactttgactac

SEQ ID NO: 118 - DNA, 48 bp, synthetic construct
  source 1..48: mol_type = other DNA
agatctagtcagagccttgtacatagtaatggaatcacctatttagag

SEQ ID NO: 119 - DNA, 21 bp, synthetic construct
  source 1..21: mol_type = other DNA
agagtttccaaccgattttct

SEQ ID NO: 120 - DNA, 27 bp, synthetic construct
  source 1..27: mol_type = other DNA
tttcaaggttcacatggtccgtacacg